European Patent Specification EP 3 486 332 B1, published April 26, 2023. Title: NUCLEIC ACIDS FOR NUCLEIC ACID AMPLIFICATION. Applicant: Becton, Dickinson, and Company. The sequence listing filed with the application follows.

SEQUENCE LISTING (16 sequences)

SEQ ID NO: 1 - DNA, 200 bp, Artificial Sequence
  Synthetic DNA
gatgctcccttcggcatccattaacctggcactcaccttgcgtatagcaggatctagccgtgtgcccgcttcgcaggcaattgaagcagagctgatgcctcttcacattgctccacctttcctgtggcgaagctccaataaattttctgcagttcaatatttcatgctgtcctccacaaatgggacaacctccatgccga

SEQ ID NO: 2 - DNA, 31 bp, Artificial Sequence
  Synthetic DNA
tgatgcctcttcacattgctccacctttcct

SEQ ID NO: 3 - DNA, 21 bp, Artificial Sequence
  Synthetic DNA
ggatctagccgtgtgcccgct

SEQ ID NO: 4 - DNA, 24 bp, Artificial Sequence
  Synthetic DNA
ggcatggaggttgtcccatttgtg

SEQ ID NO: 5 - DNA, 20 bp, Artificial Sequence
  Synthetic DNA
atctagccgtgtgcccgctt

SEQ ID NO: 6 - DNA, 25 bp, Artificial Sequence
  Synthetic DNA
ggttgtcccatttgtggaggacagc

SEQ ID NO: 7 - DNA, 3150 bp, Artificial Sequence
  Synthetic DNA
tcgttgggaaccggagctgaatgaagccataccaaacgacgagcgtgacaccacgatgcctgtagcaatggcaacaacgttgcgcaaactattaactggcgaactacttactctagcttcccggcaacaattaatagactggatggaggcggataaagttgcaggaccacttctgcgctcggcccttccggctggctggtttattgctgataaatctggagccggtgagcgtggttctcgcggtatcattgcagcactggggccagatggtaagccctcccgtatcgtagttatctacacgacggggagtcaggcaactatggatgaacgaaatagacagatcgctgagataggtgcctcactgattaagcattggtaactgtcagaccaagtttactcatatatactttagattgatttaaaacttcatttttaatttaaaaggatctaggtgaagatcctttttgataatctcatgaccaaaatcccttaacgtgagttttcgttccactgagcgtcagaccccgtagaaaagatcaaaggatcttcttgagatcctttttttctgcgcgtaatctgctgcttgcaaacaaaaaaaccaccgctaccagcggtggtttgtttgccggatcaagagctaccaactctttttccgaaggtaactggcttcagcagagcgcagataccaaatactgttcttctagtgtagccgtagttaggccaccacttcaagaactctgtagcaccgcctacatacctcgctctgctaatcctgttaccagtggctgctgccagtggcgataagtcgtgtcttaccgggttggactcaagacgatagttaccggataaggcgcagcggtcgggctgaacggggggttcgtgcacacagcccagcttggagcgaacgacctacaccgaactgagatacctacagcgtgagctatgagaaagcgccacgcttcccgaagggagaaaggcggacaggtatccggtaagcggcagggtcggaacaggagagcgcacgagggagcttccagggggaaacgcctggtatctttatagtcctgtcgggtttcgccacctctgacttgagcgtcgatttttgtgatgctcgtcaggggggcggagcctatggaaaaacgccagcaacgcggcctttttacggttcctggccttttgctggccttttgctcacatgttctttcctgcgttatcccctgattctgtggataaccgtattaccgcctttgagtgagctgataccgctcgccgcagccgaacgaccgagcgcagcgagtcagtgagcgaggaagcggaagagcgcccaatacgcaaaccgcctctccccgcgcgttggccgattcattaatgcagctggcacgacaggtttcccgactggaaagcgggcagtgagcgcaacgcaattaatgtgagttagctcactcattaggcaccccaggctttacactttatgcttccggctcgtatgttgtgtggaattgtgagcggataacaatttcacacaggaaacagctatgaccatgattacgccaagcttggatcctatctcctttcgaaagttgagaccatggaattcactggccgtcgttttacaacgtcgtgactgggaaaaccctggcgttacccaacttaatcgccttgcagcacatccccctttcgccagctggcgtaatagcgaagaggcccgcaccgatcgcccttcccaacagttgcgcagcctgaatggcgaatggcgcctgatgcggtattttctccttacgcatctgtgcggtatttcacaccgcatacgtcaaagcaaccatagtacgcgccctgtagcggcgcattaagcgcggcgggtgtggtggttacgcgcagcgtgaccgctacacttgccagcgccctagcgcccgctcctttcgctttcttcccttcctttctcgccacgttcgccggctttccccgtcaagctctaaatcgggggctccctttagggttccgatttagtgctttacggcacctcgaccccaaaaaacttgatttgggtgatggttcacgtagtgggccatcgccctgatagacggtttttcgccctttgacgttggagtccacgttctttaatagtggactcttgttccaaactggaacaacactcaaccctatctcgggctattcttttgatttataagggattttgccgatttcggcctattggttaaaaaatgagctgatttaacaaaaatttaacgcgaattttaacaaaatattaacgtttacaattttatggtgcactctcagtacaatctgctctgatgccgcatagttaagccagccccgacacccgccaacacccgctgacgcgccctgacgggcttgtctgctcccggcatccgcttacagacaagctgtgaccgtcaacgggagctgcatgtgtcagaggttttcaccgtcatcaccgaaacgcgcgacccgaaagggcctcgtgatacgcctatttttataggttaatgtcatgataataatggtttcttagacgtcaggtggcacttttcggggaaatgtgcgcggaacccctatttgtttatttttctaaatacattcaaatatgtatccgctcatgagacaataaccctgataaatgcttcaataatattgaaaaaggaagagtatgagtattcaacatttccgtgtcgcccttattcccttttttgcggcattttgccttcctgtttttgctcacccagaaacgctggtgaaagtaaaagatgctgaagatcagttgggtgcacgagtgggttacatcgaactggatctcaacagcggtaagatccttgagagttttcgccccgaagaacgttttccaatgatgagcacttttaaagttctgctatgtggcgcggtattatcccgtattgacgccgggcaagagcaactcggtcgccgcatacactattctcagaatgacttggttgagtactcaccagtcacagaaaagcatcttacggatggcatgacagtaagagaattatgcagtgctgccataaccatgagtgataacactgcggccaacttacttctgacaacgatcggaggaccgaaggagctaaccgcttttttgcacaacatgggggatcatgtaactcgccttga

SEQ ID NO: 8 - DNA, 3350 bp, Artificial Sequence
  Synthetic DNA
tcgttgggaaccggagctgaatgaagccataccaaacgacgagcgtgacaccacgatgcctgtagcaatggcaacaacgttgcgcaaactattaactggcgaactacttactctagcttcccggcaacaattaatagactggatggaggcggataaagttgcaggaccacttctgcgctcggcccttccggctggctggtttattgctgataaatctggagccggtgagcgtggttctcgcggtatcattgcagcactggggccagatggtaagccctcccgtatcgtagttatctacacgacggggagtcaggcaactatggatgaacgaaatagacagatcgctgagataggtgcctcactgattaagcattggtaactgtcagaccaagtttactcatatatactttagattgatttaaaacttcatttttaatttaaaaggatctaggtgaagatcctttttgataatctcatgaccaaaatcccttaacgtgagttttcgttccactgagcgtcagaccccgtagaaaagatcaaaggatcttcttgagatcctttttttctgcgcgtaatctgctgcttgcaaacaaaaaaaccaccgctaccagcggtggtttgtttgccggatcaagagctaccaactctttttccgaaggtaactggcttcagcagagcgcagataccaaatactgttcttctagtgtagccgtagttaggccaccacttcaagaactctgtagcaccgcctacatacctcgctctgctaatcctgttaccagtggctgctgccagtggcgataagtcgtgtcttaccgggttggactcaagacgatagttaccggataaggcgcagcggtcgggctgaacggggggttcgtgcacacagcccagcttggagcgaacgacctacaccgaactgagatacctacagcgtgagctatgagaaagcgccacgcttcccgaagggagaaaggcggacaggtatccggtaagcggcagggtcggaacaggagagcgcacgagggagcttccagggggaaacgcctggtatctttatagtcctgtcgggtttcgccacctctgacttgagcgtcgatttttgtgatgctcgtcaggggggcggagcctatggaaaaacgccagcaacgcggcctttttacggttcctggccttttgctggccttttgctcacatgttctttcctgcgttatcccctgattctgtggataaccgtattaccgcctttgagtgagctgataccgctcgccgcagccgaacgaccgagcgcagcgagtcagtgagcgaggaagcggaagagcgcccaatacgcaaaccgcctctccccgcgcgttggccgattcattaatgcagctggcacgacaggtttcccgactggaaagcgggcagtgagcgcaacgcaattaatgtgagttagctcactcattaggcaccccaggctttacactttatgcttccggctcgtatgttgtgtggaattgtgagcggataacaatttcacacaggaaacagctatgaccatgattacgccaagcttggatcctatctcctttcgatgctcccttcggcatccattaacctggcactcaccttgcgtatagcaggatctagccgtgtgcccgcttcgcaggcaattgaagcagagctgatgcctcttcacattgctccacctttcctgtggcgaagctccaataaattttctgcagttcaatatttcatgctgtcctccacaaatgggacaacctccatgccgagaaagttgagaccatggaattcactggccgtcgttttacaacgtcgtgactgggaaaaccctggcgttacccaacttaatcgccttgcagcacatccccctttcgccagctggcgtaatagcgaagaggcccgcaccgatcgcccttcccaacagttgcgcagcctgaatggcgaatggcgcctgatgcggtattttctccttacgcatctgtgcggtatttcacaccgcatacgtcaaagcaaccatagtacgcgccctgtagcggcgcattaagcgcggcgggtgtggtggttacgcgcagcgtgaccgctacacttgccagcgccctagcgcccgctcctttcgctttcttcccttcctttctcgccacgttcgccggctttccccgtcaagctctaaatcgggggctccctttagggttccgatttagtgctttacggcacctcgaccccaaaaaacttgatttgggtgatggttcacgtagtgggccatcgccctgatagacggtttttcgccctttgacgttggagtccacgttctttaatagtggactcttgttccaaactggaacaacactcaaccctatctcgggctattcttttgatttataagggattttgccgatttcggcctattggttaaaaaatgagctgatttaacaaaaatttaacgcgaattttaacaaaatattaacgtttacaattttatggtgcactctcagtacaatctgctctgatgccgcatagttaagccagccccgacacccgccaacacccgctgacgcgccctgacgggcttgtctgctcccggcatccgcttacagacaagctgtgaccgtcaacgggagctgcatgtgtcagaggttttcaccgtcatcaccgaaacgcgcgacccgaaagggcctcgtgatacgcctatttttataggttaatgtcatgataataatggtttcttagacgtcaggtggcacttttcggggaaatgtgcgcggaacccctatttgtttatttttctaaatacattcaaatatgtatccgctcatgagacaataaccctgataaatgcttcaataatattgaaaaaggaagagtatgagtattcaacatttccgtgtcgcccttattcccttttttgcggcattttgccttcctgtttttgctcacccagaaacgctggtgaaagtaaaagatgctgaagatcagttgggtgcacgagtgggttacatcgaactggatctcaacagcggtaagatccttgagagttttcgccccgaagaacgttttccaatgatgagcacttttaaagttctgctatgtggcgcggtattatcccgtattgacgccgggcaagagcaactcggtcgccgcatacactattctcagaatgacttggttgagtactcaccagtcacagaaaagcatcttacggatggcatgacagtaagagaattatgcagtgctgccataaccatgagtgataacactgcggccaacttacttctgacaacgatcggaggaccgaaggagctaaccgcttttttgcacaacatgggggatcatgtaactcgccttga

SEQ ID NO: 9 - DNA, 149 bp, Drosophila melanogaster
ggatctagccgtgtgcccgcttcgcaggcaattgaagcagagctgatgcctcttcacattgctccacctttcctgtggcgaagctccaataaattttctgcagttcaatatttcatgctgtcctccacaaatgggacaacctccatgcc

SEQ ID NO: 10 - DNA, 149 bp, Drosophila melanogaster
ggatctagccgtgtgcccgcttcgcaggcaattgaagcagagccgatgcctcttcacattgctccacctttcctgtggcgaagctccaataaattttctgcagttcaatatttcatgctgtcctccacaaatgggacaacctccatgcc

SEQ ID NO: 11 - DNA, 149 bp, Drosophila melanogaster
ggatctagccgtgtgcccgcttcgcaggcaattgaagcagagccgatgcctcttcacattgctccacctttcctgtggcgaagctccaataaattttctgcagttcaatatttcatgctgtcctccacagatgggacaacctccatgcc

SEQ ID NO: 12 - DNA, 149 bp, Drosophila melanogaster
ggatctagccgtgtgcccgcttcgcaggcaattgaagcagagccgatgcctcttcacattgctccacctttcctgtgccgaagctccaataaattttctgcagttcaatatttcatgctgtcctccacagatgggacaacctccatgcc

SEQ ID NO: 13 - DNA, 149 bp, Drosophila melanogaster; identical to SEQ ID NO: 12

SEQ ID NO: 14 - DNA, 200 bp, Drosophila melanogaster
gatgctcccttcggcatccattaacctggcactcaccttgcgtatagcaggatctagccgtgtgcccgcttcgcaggcaattgaagcagagccgatgcctcttcacattgctccacctttcctgtggcgaagctccaataaattttctgcagttcaatatttcatgctgtcctccacaaatgggacaacctccatgccga

SEQ ID NO: 15 - DNA, 3350 bp, Artificial Sequence
  Synthetic DNA
tcgttgggaaccggagctgaatgaagccataccaaacgacgagcgtgacaccacgatgcctgtagcaatggcaacaacgttgcgcaaactattaactggcgaactacttactctagcttcccggcaacaattaatagactggatggaggcggataaagttgcaggaccacttctgcgctcggcccttccggctggctggtttattgctgataaatctggagccggtgagcgtggttctcgcggtatcattgcagcactggggccagatggtaagccctcccgtatcgtagttatctacacgacggggagtcaggcaactatggatgaacgaaatagacagatcgctgagataggtgcctcactgattaagcattggtaactgtcagaccaagtttactcatatatactttagattgatttaaaacttcatttttaatttaaaaggatctaggtgaagatcctttttgataatctcatgaccaaaatcccttaacgtgagttttcgttccactgagcgtcagaccccgtagaaaagatcaaaggatcttcttgagatcctttttttctgcgcgtaatctgctgcttgcaaacaaaaaaaccaccgctaccagcggtggtttgtttgccggatcaagagctaccaactctttttccgaaggtaactggcttcagcagagcgcagataccaaatactgttcttctagtgtagccgtagttaggccaccacttcaagaactctgtagcaccgcctacatacctcgctctgctaatcctgttaccagtggctgctgccagtggcgataagtcgtgtcttaccgggttggactcaagacgatagttaccggataaggcgcagcggtcgggctgaacggggggttcgtgcacacagcccagcttggagcgaacgacctacaccgaactgagatacctacagcgtgagctatgagaaagcgccacgcttcccgaagggagaaaggcggacaggtatccggtaagcggcagggtcggaacaggagagcgcacgagggagcttccagggggaaacgcctggtatctttatagtcctgtcgggtttcgccacctctgacttgagcgtcgatttttgtgatgctcgtcaggggggcggagcctatggaaaaacgccagcaacgcggcctttttacggttcctggccttttgctggccttttgctcacatgttctttcctgcgttatcccctgattctgtggataaccgtattaccgcctttgagtgagctgataccgctcgccgcagccgaacgaccgagcgcagcgagtcagtgagcgaggaagcggaagagcgcccaatacgcaaaccgcctctccccgcgcgttggccgattcattaatgcagctggcacgacaggtttcccgactggaaagcgggcagtgagcgcaacgcaattaatgtgagttagctcactcattaggcaccccaggctttacactttatgcttccggctcgtatgttgtgtggaattgtgagcggataacaatttcacacaggaaacagctatgaccatgattacgccaagcttggatcctatctcctttcgatgctcccttcggcatccattaacctggcactcaccttgcgtatagcaggatctagccgtgtgcccgcttcgcaggcaattgaagcagagccgatgcctcttcacattgctccacctttcctgtggcgaagctccaataaattttctgcagttcaatatttcatgctgtcctccacaaatgggacaacctccatgccgagaaagttgagaccatggaattcactggccgtcgttttacaacgtcgtgactgggaaaaccctggcgttacccaacttaatcgccttgcagcacatccccctttcgccagctggcgtaatagcgaagaggcccgcaccgatcgcccttcccaacagttgcgcagcctgaatggcgaatggcgcctgatgcggtattttctccttacgcatctgtgcggtatttcacaccgcatacgtcaaagcaaccatagtacgcgccctgtagcggcgcattaagcgcggcgggtgtggtggttacgcgcagcgtgaccgctacacttgccagcgccctagcgcccgctcctttcgctttcttcccttcctttctcgccacgttcgccggctttccccgtcaagctctaaatcgggggctccctttagggttccgatttagtgctttacggcacctcgaccccaaaaaacttgatttgggtgatggttcacgtagtgggccatcgccctgatagacggtttttcgccctttgacgttggagtccacgttctttaatagtggactcttgttccaaactggaacaacactcaaccctatctcgggctattcttttgatttataagggattttgccgatttcggcctattggttaaaaaatgagctgatttaacaaaaatttaacgcgaattttaacaaaatattaacgtttacaattttatggtgcactctcagtacaatctgctctgatgccgcatagttaagccagccccgacacccgccaacacccgctgacgcgccctgacgggcttgtctgctcccggcatccgcttacagacaagctgtgaccgtcaacgggagctgcatgtgtcagaggttttcaccgtcatcaccgaaacgcgcgacccgaaagggcctcgtgatacgcctatttttataggttaatgtcatgataataatggtttcttagacgtcaggtggcacttttcggggaaatgtgcgcggaacccctatttgtttatttttctaaatacattcaaatatgtatccgctcatgagacaataaccctgataaatgcttcaataatattgaaaaaggaagagtatgagtattcaacatttccgtgtcgcccttattcccttttttgcggcattttgccttcctgtttttgctcacccagaaacgctggtgaaagtaaaagatgctgaagatcagttgggtgcacgagtgggttacatcgaactggatctcaacagcggtaagatccttgagagttttcgccccgaagaacgttttccaatgatgagcacttttaaagttctgctatgtggcgcggtattatcccgtattgacgccgggcaagagcaactcggtcgccgcatacactattctcagaatgacttggttgagtactcaccagtcacagaaaagcatcttacggatggcatgacagtaagagaattatgcagtgctgccataaccatgagtgataacactgcggccaacttacttctgacaacgatcggaggaccgaaggagctaaccgcttttttgcacaacatgggggatcatgtaactcgccttga

SEQ ID NO: 16 - DNA, 32 bp, Artificial Sequence
  Synthetic DNA
ttgatgcctcttcacattgctccacctttcct